European Patent Application EP 4 450 489 A1, published October 23, 2024. Title: Improved Oxazalines Click Reaction. Applicant: Synaffix B.V. The sequence listing filed with the application follows.

SEQUENCE LISTING (19 sequences)

SEQ ID NO: 1 - protein, 26 aa, synthetic construct
  source 1..26: note = protease-cleavable linker 1
GSSGGSGGSGGSGLSGRSDNHGSSGS

SEQ ID NO: 2 - protein, 18 aa, synthetic construct
  source 1..18: note = protease-cleavable linker 2
GGGGSGGGGSRASRANGS

SEQ ID NO: 3 - protein, 114 aa, Homo sapiens
  source 1..114: note = human IL-15
NWVNVISDLKKIEDLIQSMHIDATLYTESDVHPSCKVTAMKCFLLELQVISLESGDASIHDTVENLIILANNSLSSNGNVTESGCKECEELEEKNIKEFLQSFVHIVQMFINTS

SEQ ID NO: 4 - protein, 211 aa, synthetic construct
  source 1..211: note = IL-15Ra-IL-15 fusion protein
ITCPPPMSVEHADIWVKSYSLYSRERYICNSGFKRKAGTSSLTECVLNKATNVAHWTTPSLKCIRDPALVHQRPAPPSGGSGGGGSGGGSGGGGSLQNWVNVISDLKKIEDLIQSMHIDATLYTESDVHPSCKVTAMKCFLLELQVISLESGDASIHDTVENLIILANNSLSSNGNVTESGCKECEELEEKNIKEFLQSFVHIVQMFINTS

SEQ ID NO: 5 - protein, 136 aa, synthetic construct
  source 1..136: note = SYR-cleavable linker 2-IL15 (PF51)
MSYRGGGGSGGGGSRASRANGSNWVNVISDLKKIEDLIQSMHIDATLYTESDVHPSCKVTAMKCFLLELQVISLESGDASIHDTVENLIILANNSLSSNGNVTESGCKECEELEEKNIKEFLQSFVHIVQMFINTS

SEQ ID NO: 6 - protein, 132 aa, synthetic construct
  source 1..132: note = ST-cleavable linker 2-IL15 (PF52)
STGGGGSGGGGSRASRANGSNWVNVISDLKKIEDLIQSMHIDATLYTESDVHPSCKVTAMKCFLLELQVISLESGDASIHDTVENLIILANNSLSSNGNVTESGCKECEELEEKNIKEFLQSFVHIVQMFIN

SEQ ID NO: 7 - protein, 255 aa, synthetic construct
  source 1..255: note = SYR-(G4S)8-IL15Ra-IL-15 (PF57)
MSYRGGGGSGGGGSGGGGSGGGGSGGGGSGGGGSGGGGSGGGGSITCPPPMSVEHADIWVKSYSLYSRERYICNSGFKRKAGTSSLTECVLNKATNVAHWTTPSLKCIRDPALVHQRPAPPSGGSGGGGSGGGSGGGGSLQNWVNVISDLKKIEDLIQSMHIDATLYTESDVHPSCKVTAMKCFLLELQVISLESGDASIHDTVENLIILANNSLSSNGNVTESGCKECEELEEKNIKEFLQSFVHIVQMFINTS

SEQ ID NO: 8 - protein, 252 aa, synthetic construct
  source 1..252: note = S-(G4S)8-IL15Ra-IL-15 (PF58)
SGGGGSGGGGSGGGGSGGGGSGGGGSGGGGSGGGGSGGGGSITCPPPMSVEHADIWVKSYSLYSRERYICNSGFKRKAGTSSLTECVLNKATNVAHWTTPSLKCIRDPALVHQRPAPPSGGSGGGGSGGGSGGGGSLQNWVNVISDLKKIEDLIQSMHIDATLYTESDVHPSCKVTAMKCFLLELQVISLESGDASIHDTVENLIILANNSLSSNGNVTESGCKECEELEEKNIKEFLQSFVHIVQMFINTS

SEQ ID NO: 9 - protein, 252 aa, synthetic construct
  source 1..252: note = ST-(G4S)8-IL15Ra-IL-15 (PF59)
STGGGGSGGGGSGGGGSGGGGSGGGGSGGGGSGGGGSGGGGSITCPPPMSVEHADIWVKSYSLYSRERYICNSGFKRKAGTSSLTECVLNKATNVAHWTTPSLKCIRDPALVHQRPAPPSGGSGGGGSGGGSGGGGSLQNWVNVISDLKKIEDLIQSMHIDATLYTESDVHPSCKVTAMKCFLLELQVISLESGDASIHDTVENLIILANNSLSSNGNVTESGCKECEELEEKNIKEFLQSFVHIVQMFINT

SEQ ID NO: 10 - protein, 215 aa, synthetic construct
  source 1..215: note = mPD-L1 light chain
QSALTQPASVSGSPGQSITISCTGTSSDVGAYNYVSWYQQHPGKAPKLMIYDVSNRPSGVSNRFSGSKSGNTASLTISGLQAEDEADYYCSSYTSSSTRVFGTGTKVTVLGQPKANPTVTLFPPSSEELQANKATLVCLISDFYPGAVTVAWKADGSPVKAGVETTKPSKQSNNKYAASSYLSLTPEQWKSHRSYSCQVTHEGSTVEKTVAPTEC

SEQ ID NO: 11 - protein, 450 aa, synthetic construct
  source 1..450: note = mPD-L1 heavy chain
EVQLLESGGGLVQPGGSLRLSCAASGFTFSAYRMFWVRQAPGKGLEWVSSIYPSGGITFYADSVKGRFTISRDNSKNTLYLQMNSLRAEDTAIYYCARIKLGTVTTVDYWGQGTLVTVSSASTKGPSVFPLAPSSKSTSGGTAALGCLVKDYFPEPVTVSWNSGALTSGVHTFPAVLQSSGLYSLSSVVTVPSSSLGTQTYICNVNHKPSNTKVDKRVEPKSCDKTHTCPPCPAPELLGGPSVFLFPPKPKDTLMISRTPEVTCVVVDVSHEDPEVKFNWYVDGVEVHNAKTKPREEQYNSTYRVVSVLTVLHQDWLNGKEYKCKVSNKALPAPIEKTISKAKGQPREPQVYTLPPSREEMTKNQVSLTCLVKGFYPSDIAVEWESNGQPENNYKTTPPVLDSDGSFFLYSKLTVDKSRWQQGNVFSCSVMHEALHNHYTQKSLSLSPGK

SEQ ID NO: 12 - protein, 4 aa, synthetic construct
  source 1..4: note = peptide spacer 1
GGGG

SEQ ID NO: 13 - protein, 4 aa, synthetic construct
  source 1..4: note = peptide spacer 2
GGFG

SEQ ID NO: 14 - protein, 4 aa, synthetic construct
  source 1..4: note = peptide spacer 3
GFGG

SEQ ID NO: 15 - protein, 4 aa, synthetic construct
  source 1..4: note = peptide spacer 4
FGGG

SEQ ID NO: 16 - protein, 4 aa, synthetic construct
  source 1..4: note = peptide spacer 5
GGGF

SEQ ID NO: 17 - protein, 4 aa, synthetic construct
  source 1..4: note = peptide spacer 6
FFGG

SEQ ID NO: 18 - protein, 4 aa, synthetic construct
  source 1..4: note = peptide spacer 7
GGFF

SEQ ID NO: 19 - protein, 5 aa, synthetic construct
  source 1..5: note = peptide spacer 8
GGGFG